European Patent Application EP 4 659 765 A2, published December 10, 2025. Title: DYSTROPHIN GENE EXON DELEATION USING ENGINEERED NUCLEASES. Applicant: Precision Biosciences, Inc. Application EP 25191909.8, filed March 12, 2015. The sequence listing filed with the application follows.

SEQUENCE LISTING (188 sequences)

SEQ ID NO: 1 - protein, 163 aa, Chlamydomonas reinhardtii
MNTKYNKEFLLYLAGFVDGDGSIIAQIKPNQSYKFKHQLSLAFQVTQKTQRRWFLDKLVDEIGVGYVRDRGSVSDYILSEIKPLHNFLTQLQPFLKLKQKQANLVLKIIWRLPSAKESPDKFLEVCTWVDQIAALNDSKTRKTTSETVRAVLDSLSEKKKSSP

SEQ ID NO: 2 - DNA, 22 bp, Homo sapiens
  source 1..22: mol_type = genomic DNA
ttctctgtggtgagaaaattta

SEQ ID NO: 3 - DNA, 22 bp, Homo sapiens
  source 1..22: mol_type = genomic DNA
ttcactattttgaaatatacag

SEQ ID NO: 4 - DNA, 22 bp, Homo sapiens
  source 1..22: mol_type = genomic DNA
tattttgaaatatacagcacaa

SEQ ID NO: 5 - DNA, 22 bp, Homo sapiens
  source 1..22: mol_type = genomic DNA
taactttgttcatattactatg

SEQ ID NO: 6 - DNA, 22 bp, Homo sapiens
  source 1..22: mol_type = genomic DNA
actttgttcatattactatgca

SEQ ID NO: 7 - DNA, 22 bp, Homo sapiens
  source 1..22: mol_type = genomic DNA
catattactatgcaatagaaca

SEQ ID NO: 8 - DNA, 22 bp, Homo sapiens
  source 1..22: mol_type = genomic DNA
cactagaacttattactccttt

SEQ ID NO: 9 - DNA, 22 bp, Homo sapiens
  source 1..22: mol_type = genomic DNA
tttcagttgatgaacaggcagt

SEQ ID NO: 10 - DNA, 22 bp, Homo sapiens
  source 1..22: mol_type = genomic DNA
agttttggatcaagaataatat

SEQ ID NO: 11 - DNA, 22 bp, Homo sapiens
  source 1..22: mol_type = genomic DNA
aaaaatattttgaaagggaata

SEQ ID NO: 12 - DNA, 22 bp, Homo sapiens
  source 1..22: mol_type = genomic DNA
ccaaataatttattacaatgtt

SEQ ID NO: 13 - DNA, 22 bp, Homo sapiens
  source 1..22: mol_type = genomic DNA
atctttcttttaatcaataaat

SEQ ID NO: 14 - DNA, 22 bp, Homo sapiens
  source 1..22: mol_type = genomic DNA
ttttaatcaataaatatattca

SEQ ID NO: 15 - DNA, 22 bp, Homo sapiens
  source 1..22: mol_type = genomic DNA
accttccatttaaaatcagctt

SEQ ID NO: 16 - DNA, 22 bp, Homo sapiens
  source 1..22: mol_type = genomic DNA
tcagcttttatattgagtattt

SEQ ID NO: 17 - DNA, 22 bp, Homo sapiens
  source 1..22: mol_type = genomic DNA
gcttttatattgagtatttttt

SEQ ID NO: 18 - DNA, 22 bp, Homo sapiens
  source 1..22: mol_type = genomic DNA
taaaatgttgtgtgtacatgct

SEQ ID NO: 19 - DNA, 22 bp, Homo sapiens
  source 1..22: mol_type = genomic DNA
atgttgtgtgtacatgctaggt

SEQ ID NO: 20 - DNA, 22 bp, Homo sapiens
  source 1..22: mol_type = genomic DNA
gctaggtgtgtatattaatttt

SEQ ID NO: 21 - DNA, 22 bp, Homo sapiens
  source 1..22: mol_type = genomic DNA
atttgttacttgaaactaaact

SEQ ID NO: 22 - DNA, 22 bp, Homo sapiens
  source 1..22: mol_type = genomic DNA
ctaaactctgcaaatgcaggaa

SEQ ID NO: 23 - DNA, 22 bp, Homo sapiens
  source 1..22: mol_type = genomic DNA
gtgatatctttgtcagtataac

SEQ ID NO: 24 - DNA, 22 bp, Homo sapiens
  source 1..22: mol_type = genomic DNA
aaaaaatatacgctatatctct

SEQ ID NO: 25 - DNA, 22 bp, Homo sapiens
  source 1..22: mol_type = genomic DNA
atctgttttacataatccatct

SEQ ID NO: 26 - DNA, 22 bp, Homo sapiens
  source 1..22: mol_type = genomic DNA
ctgttttacataatccatctat

SEQ ID NO: 27 - DNA, 22 bp, Homo sapiens
  source 1..22: mol_type = genomic DNA
ctatttttcttgatccatatgc

SEQ ID NO: 28 - DNA, 22 bp, Homo sapiens
  source 1..22: mol_type = genomic DNA
catatgcttttacctgcaggcg

SEQ ID NO: 29 - DNA, 22 bp, Homo sapiens
  source 1..22: mol_type = genomic DNA
aaattacttttgactgttgttg

SEQ ID NO: 30 - DNA, 22 bp, Homo sapiens
  source 1..22: mol_type = genomic DNA
tgactgttgttgtcatcattat

SEQ ID NO: 31 - DNA, 22 bp, Homo sapiens
  source 1..22: mol_type = genomic DNA
ttgttgtcatcattatattact

SEQ ID NO: 32 - DNA, 22 bp, Homo sapiens
  source 1..22: mol_type = genomic DNA
ttgtcatcattatattactaga

SEQ ID NO: 33 - DNA, 22 bp, Homo sapiens
  source 1..22: mol_type = genomic DNA
atcattatattactagaaagaa

SEQ ID NO: 34 - DNA, 22 bp, Homo sapiens
  source 1..22: mol_type = genomic DNA
aaaattatcataatgataatat

SEQ ID NO: 35 - DNA, 22 bp, Homo sapiens
  source 1..22: mol_type = genomic DNA
atggactttttgtgtcaggatg

SEQ ID NO: 36 - DNA, 22 bp, Homo sapiens
  source 1..22: mol_type = genomic DNA
ggactttttgtgtcaggatgag

SEQ ID NO: 37 - DNA, 22 bp, Homo sapiens
  source 1..22: mol_type = genomic DNA
ggagctggtttatctgataaac

SEQ ID NO: 38 - DNA, 22 bp, Homo sapiens
  source 1..22: mol_type = genomic DNA
attgaatctgtgacagagggaa

SEQ ID NO: 39 - DNA, 22 bp, Homo sapiens
  source 1..22: mol_type = genomic DNA
agggaagcatcgtaacagcaag

SEQ ID NO: 40 - DNA, 22 bp, Homo sapiens
  source 1..22: mol_type = genomic DNA
gggcagtgtgtatttcggcttt

SEQ ID NO: 41 - DNA, 22 bp, Homo sapiens
  source 1..22: mol_type = genomic DNA
tatattctattgacaaaatgcc

SEQ ID NO: 42 - DNA, 22 bp, Homo sapiens
  source 1..22: mol_type = genomic DNA
taattgttggtacttattgaca

SEQ ID NO: 43 - DNA, 22 bp, Homo sapiens
  source 1..22: mol_type = genomic DNA
tgttggtacttattgacatttt

SEQ ID NO: 44 - DNA, 22 bp, Homo sapiens
  source 1..22: mol_type = genomic DNA
ttttatggtttatgttaatagg

SEQ ID NO: 45 - DNA, 22 bp, Homo sapiens
  source 1..22: mol_type = genomic DNA
agtttttttttaatactgtgac

SEQ ID NO: 46 - DNA, 22 bp, Homo sapiens
  source 1..22: mol_type = genomic DNA
tttaatactgtgactaacctat

SEQ ID NO: 47 - DNA, 22 bp, Homo sapiens
  source 1..22: mol_type = genomic DNA
tttcacctctcgtatccacgat

SEQ ID NO: 48 - DNA, 22 bp, Homo sapiens
  source 1..22: mol_type = genomic DNA
tcacctctcgtatccacgatca

SEQ ID NO: 49 - DNA, 22 bp, Homo sapiens
  source 1..22: mol_type = genomic DNA
ctcgtatccacgatcactaaga

SEQ ID NO: 50 - DNA, 22 bp, Homo sapiens
  source 1..22: mol_type = genomic DNA
ccaaatactttgttcatgttta

SEQ ID NO: 51 - DNA, 22 bp, Homo sapiens
  source 1..22: mol_type = genomic DNA
ggaacatccttgtggggacaag

SEQ ID NO: 52 - DNA, 22 bp, Homo sapiens
  source 1..22: mol_type = genomic DNA
aatttgctcttgaaaaggtttc

SEQ ID NO: 53 - DNA, 22 bp, Homo sapiens
  source 1..22: mol_type = genomic DNA
ctaattgatttgtaggacatta

SEQ ID NO: 54 - DNA, 22 bp, Homo sapiens
  source 1..22: mol_type = genomic DNA
ttccctgacacataaaaggtgt

SEQ ID NO: 55 - DNA, 22 bp, Homo sapiens
  source 1..22: mol_type = genomic DNA
ccctgacacataaaaggtgtct

SEQ ID NO: 56 - DNA, 22 bp, Homo sapiens
  source 1..22: mol_type = genomic DNA
ctttctgtcttgtatcctttgg

SEQ ID NO: 57 - DNA, 22 bp, Homo sapiens
  source 1..22: mol_type = genomic DNA
atcctttggatatgggcatgtc

SEQ ID NO: 58 - DNA, 22 bp, Homo sapiens
  source 1..22: mol_type = genomic DNA
tggatatgggcatgtcagtttc

SEQ ID NO: 59 - DNA, 22 bp, Homo sapiens
  source 1..22: mol_type = genomic DNA
gatatgggcatgtcagtttcat

SEQ ID NO: 60 - DNA, 22 bp, Homo sapiens
  source 1..22: mol_type = genomic DNA
gaaattttcacatggagctttt

SEQ ID NO: 61 - DNA, 22 bp, Homo sapiens
  source 1..22: mol_type = genomic DNA
tttctttctttgccagtacaac

SEQ ID NO: 62 - DNA, 22 bp, Homo sapiens
  source 1..22: mol_type = genomic DNA
tctttgccagtacaactgcatg

SEQ ID NO: 63 - DNA, 22 bp, Homo sapiens
  source 1..22: mol_type = genomic DNA
tttggtatcttacaggaactcc

SEQ ID NO: 64 - DNA, 22 bp, Homo sapiens
  source 1..22: mol_type = genomic DNA
aagaatatttcatgagagatta

SEQ ID NO: 65 - DNA, 22 bp, Homo sapiens
  source 1..22: mol_type = genomic DNA
gaatatttcatgagagattata

SEQ ID NO: 66 - DNA, 22 bp, Homo sapiens
  source 1..22: mol_type = genomic DNA
tgagagattataagcagggtga

SEQ ID NO: 67 - DNA, 22 bp, Homo sapiens
  source 1..22: mol_type = genomic DNA
aaggcactaacattaaagaacc

SEQ ID NO: 68 - DNA, 22 bp, Homo sapiens
  source 1..22: mol_type = genomic DNA
tcaacagcagtaaagaaatttt

SEQ ID NO: 69 - DNA, 22 bp, Homo sapiens
  source 1..22: mol_type = genomic DNA
ttctttttttcatatactaaaa

SEQ ID NO: 70 - DNA, 22 bp, Homo sapiens
  source 1..22: mol_type = genomic DNA
ctaaaatatatacttgtggcta

SEQ ID NO: 71 - DNA, 22 bp, Homo sapiens
  source 1..22: mol_type = genomic DNA
tgaatatcttcaatatatttta

SEQ ID NO: 72 - DNA, 22 bp, Homo sapiens
  source 1..22: mol_type = genomic DNA
caattataaatgattgttttgt

SEQ ID NO: 73 - DNA, 22 bp, Homo sapiens
  source 1..22: mol_type = genomic DNA
atgattgttttgtaggaaagac

SEQ ID NO: 74 - DNA, 22 bp, Homo sapiens
  source 1..22: mol_type = genomic DNA
tcatattttgtacaaaataaac

SEQ ID NO: 75 - DNA, 22 bp, Homo sapiens
  source 1..22: mol_type = genomic DNA
atacgtgtattgcttgtactac

SEQ ID NO: 76 - DNA, 22 bp, Homo sapiens
  source 1..22: mol_type = genomic DNA
gtattgcttgtactactcactg

SEQ ID NO: 77 - DNA, 22 bp, Homo sapiens
  source 1..22: mol_type = genomic DNA
actgaatctacacaactgccct

SEQ ID NO: 78 - DNA, 22 bp, Homo sapiens
  source 1..22: mol_type = genomic DNA
tgaatctacacaactgccctta

SEQ ID NO: 79 - DNA, 22 bp, Homo sapiens
  source 1..22: mol_type = genomic DNA
caactgcccttatgacatttac

SEQ ID NO: 80 - DNA, 22 bp, Homo sapiens
  source 1..22: mol_type = genomic DNA
ggtaaatacatgaaaaatgctt

SEQ ID NO: 81 - DNA, 22 bp, Homo sapiens
  source 1..22: mol_type = genomic DNA
ttgccttgcttactgcttattg

SEQ ID NO: 82 - DNA, 22 bp, Homo sapiens
  source 1..22: mol_type = genomic DNA
gcttactgcttattgctagtac

SEQ ID NO: 83 - DNA, 22 bp, Homo sapiens
  source 1..22: mol_type = genomic DNA
tagtactgaacaaatgttagaa

SEQ ID NO: 84 - DNA, 22 bp, Homo sapiens
  source 1..22: mol_type = genomic DNA
actgaacaaatgttagaactga

SEQ ID NO: 85 - DNA, 22 bp, Homo sapiens
  source 1..22: mol_type = genomic DNA
aagatttatttaatgactttga

SEQ ID NO: 86 - DNA, 22 bp, Homo sapiens
  source 1..22: mol_type = genomic DNA
cagtatttcatgtctaaataga

SEQ ID NO: 87 - DNA, 22 bp, Homo sapiens
  source 1..22: mol_type = genomic DNA
ggtttttcttcactgctggcca

SEQ ID NO: 88 - DNA, 22 bp, Homo sapiens
  source 1..22: mol_type = genomic DNA
caatctgaaataaaaagaaaaa

SEQ ID NO: 89 - DNA, 22 bp, Homo sapiens
  source 1..22: mol_type = genomic DNA
ctgctcccagtataaaatacag

SEQ ID NO: 90 - DNA, 22 bp, Homo sapiens
  source 1..22: mol_type = genomic DNA
aagaacgtttcattggctttga

SEQ ID NO: 91 - DNA, 22 bp, Homo sapiens
  source 1..22: mol_type = genomic DNA
acttcctattcaagggaatttt

SEQ ID NO: 92 - DNA, 22 bp, Homo sapiens
  source 1..22: mol_type = genomic DNA
tgttttttcttgaataaaaaaa

SEQ ID NO: 93 - DNA, 22 bp, Homo sapiens
  source 1..22: mol_type = genomic DNA
ttttcttgaataaaaaaaaaat

SEQ ID NO: 94 - DNA, 22 bp, Homo sapiens
  source 1..22: mol_type = genomic DNA
ttgttttctttaccacttccac

SEQ ID NO: 95 - DNA, 22 bp, Homo sapiens
  source 1..22: mol_type = genomic DNA
acaatgtatatgattgttactg

SEQ ID NO: 96 - DNA, 22 bp, Homo sapiens
  source 1..22: mol_type = genomic DNA
tgtatatgattgttactgagaa

SEQ ID NO: 97 - DNA, 22 bp, Homo sapiens
  source 1..22: mol_type = genomic DNA
cttgtccaggcatgagaatgag

SEQ ID NO: 98 - DNA, 22 bp, Homo sapiens
  source 1..22: mol_type = genomic DNA
tgtccaggcatgagaatgagca

SEQ ID NO: 99 - DNA, 22 bp, Homo sapiens
  source 1..22: mol_type = genomic DNA
aatcgttttttaaaaaattgtt

SEQ ID NO: 100 - DNA, 22 bp, Homo sapiens
  source 1..22: mol_type = genomic DNA
ttctaccatgtattgctaaaca

SEQ ID NO: 101 - DNA, 22 bp, Homo sapiens
  source 1..22: mol_type = genomic DNA
taccatgtattgctaaacaaag

SEQ ID NO: 102 - DNA, 22 bp, Homo sapiens
  source 1..22: mol_type = genomic DNA
tataatgtcatgaataagagtt

SEQ ID NO: 103 - DNA, 22 bp, Homo sapiens
  source 1..22: mol_type = genomic DNA
atgtcatgaataagagtttggc

SEQ ID NO: 104 - DNA, 22 bp, Homo sapiens
  source 1..22: mol_type = genomic DNA
ttttcctttttgcaaaaaccca

SEQ ID NO: 105 - DNA, 22 bp, Homo sapiens
  source 1..22: mol_type = genomic DNA
ttcctttttgcaaaaacccaaa

SEQ ID NO: 106 - DNA, 22 bp, Homo sapiens
  source 1..22: mol_type = genomic DNA
agttcttaggcaactgtttctc

SEQ ID NO: 107 - DNA, 22 bp, Homo sapiens
  source 1..22: mol_type = genomic DNA
tctctctcagcaaacacattac

SEQ ID NO: 108 - DNA, 22 bp, Homo sapiens
  source 1..22: mol_type = genomic DNA
taagtataatcaaggatataaa

SEQ ID NO: 109 - DNA, 22 bp, Homo sapiens
  source 1..22: mol_type = genomic DNA
agtagccatacattaaaaagga

SEQ ID NO: 110 - DNA, 22 bp, Homo sapiens
  source 1..22: mol_type = genomic DNA
aggaaatatacaaaaaaaaaaa

SEQ ID NO: 111 - DNA, 22 bp, Homo sapiens
  source 1..22: mol_type = genomic DNA
agaaaccttacaagaatagttg

SEQ ID NO: 112 - DNA, 22 bp, Homo sapiens
  source 1..22: mol_type = genomic DNA
caagaatagttgtctcagttaa

SEQ ID NO: 113 - DNA, 22 bp, Homo sapiens
  source 1..22: mol_type = genomic DNA
atctattttataccaaataagt

SEQ ID NO: 114 - DNA, 22 bp, Homo sapiens
  source 1..22: mol_type = genomic DNA
ttataccaaataagtcactcaa

SEQ ID NO: 115 - DNA, 22 bp, Homo sapiens
  source 1..22: mol_type = genomic DNA
tttgttttggcactacgcagcc

SEQ ID NO: 116 - DNA, 22 bp, Homo sapiens
  source 1..22: mol_type = genomic DNA
taaggataattgaaagagagct

SEQ ID NO: 117 - DNA, 22 bp, Homo sapiens
  source 1..22: mol_type = genomic DNA
agaaaagtaacaaaacataaga

SEQ ID NO: 118 - DNA, 22 bp, Homo sapiens
  source 1..22: mol_type = genomic DNA
ttaaagttggcatttatgcaat

SEQ ID NO: 119 - DNA, 22 bp, Homo sapiens
  source 1..22: mol_type = genomic DNA
agttggcatttatgcaatgcca

SEQ ID NO: 120 - DNA, 22 bp, Homo sapiens
  source 1..22: mol_type = genomic DNA
aacatgtttttaatacaaatag

SEQ ID NO: 121 - DNA, 22 bp, Homo sapiens
  source 1..22: mol_type = genomic DNA
tacattgatgtaaatatggttt

SEQ ID NO: 122 - DNA, 22 bp, Homo sapiens
  source 1..22: mol_type = genomic DNA
atatcttttatatttgtgaatg

SEQ ID NO: 123 - DNA, 22 bp, Homo sapiens
  source 1..22: mol_type = genomic DNA
cttttatatttgtgaatgatta

SEQ ID NO: 124 - DNA, 22 bp, Homo sapiens
  source 1..22: mol_type = genomic DNA
tgtgaatgattaagaaaaataa

SEQ ID NO: 125 - DNA, 22 bp, Homo sapiens
  source 1..22: mol_type = genomic DNA
aattgttatacattaaagtttt

SEQ ID NO: 126 - DNA, 22 bp, Homo sapiens
  source 1..22: mol_type = genomic DNA
aaagttttttcacttgtaacag

SEQ ID NO: 127 - DNA, 22 bp, Homo sapiens
  source 1..22: mol_type = genomic DNA
taacagctttcaagcctttcta

SEQ ID NO: 128 - DNA, 22 bp, Homo sapiens
  source 1..22: mol_type = genomic DNA
ggtatttaggtattaaagtact

SEQ ID NO: 129 - DNA, 22 bp, Homo sapiens
  source 1..22: mol_type = genomic DNA
tactaccttttgaaaaaacaag

SEQ ID NO: 130 - DNA, 22 bp, Homo sapiens
  source 1..22: mol_type = genomic DNA
ggaatttctttgtaaaataaac

SEQ ID NO: 131 - DNA, 22 bp, Homo sapiens
  source 1..22: mol_type = genomic DNA
aacctgcatttaaaggccttga

SEQ ID NO: 132 - DNA, 22 bp, Homo sapiens
  source 1..22: mol_type = genomic DNA
tgagcttgaatacagaagacct

SEQ ID NO: 133 - DNA, 22 bp, Homo sapiens
  source 1..22: mol_type = genomic DNA
tgattgtggtcaagccatctct

SEQ ID NO: 134 - DNA, 22 bp, Homo sapiens
  source 1..22: mol_type = genomic DNA
ctattctgagtacagagcatac

SEQ ID NO: 135 - protein, 364 aa, synthetic construct
  REGION 1..364: note = Description of Artificial Sequence: Syntheticpolypeptide
MAPKKKRKVHMNTKYNKEFLLYLAGFVDGDGSIYAWISPSQTCKFKHRLMLRFIVSQKTQRRWFLDKLVDEIGVGYVQDCGSVSEYRLSEIKPLHNFLTQLQPFLKLKQKQANLVLKIIEQLPSAKESPDKFLEVCTWVDQIAALNDSKTRKTTSETVRAVLDSLPGSVGGLSPSQASSAASSASSSPGSGISEALRAGAGSGTGYNKEFLLYLAGFVDGDGSIYACILPTQRQKFKHGLTLYFRVTQKTQRRWFLDKLVDEIGVGYVLDFGSVSCYSLSQIKPLHNFLTQLQPFLKLKQKQANLVLKIIEQLPSAKESPDKFLEVCTWVDQIAALNDSKTRKTTSETVRAVLDSLSEKKKSSP

SEQ ID NO: 136 - protein, 364 aa, synthetic construct
  REGION 1..364: note = Description of Artificial Sequence: Syntheticpolypeptide
MAPKKKRKVHMNTKYNKEFLLYLAGFVDGDGSIFASIRPRQTSKFKHALALFFVVGQKTQRRWFLDKLVDEIGVGYVYDRGSVSVYQLSQIKPLHNFLTQLQPFLKLKQKQANLVLKIIEQLPSAKESPDKFLEVCTWVDQIAALNDSKTRKTTSETVRAVLDSLPGSVGGLSPSQASSAASSASSSPGSGISEALRAGAGSGTGYNKEFLLYLAGFVDGDGSIIACIRPHQAYKFKHQLCLSFCVYQKTQRRWFLDKLVDEIGVGYVTDAGSVSSYRLSEIKPLHNFLTQLQPFLKLKQKQANLVLKIIEQLPSAKESPDKFLEVCTWVDQIAALNDSKTRKTTSETVRAVLDSLSEKKKSSP

SEQ ID NO: 137 - protein, 364 aa, synthetic construct
  REGION 1..364: note = Description of Artificial Sequence: Syntheticpolypeptide
MAPKKKRKVHMNTKYNKEFLLYLAGFVDGDGSIFACIQPDQRAKFKHTLRLSFEVGQKTQRRWFLDKLVDEIGVGYVNDSGSVSKYRLSQIKPLHNFLTQLQPFLKLKQKQANLVLKIIEQLPSAKESPDKFLEVCTWVDQIAALNDSKTRKTTSETVRAVLDSLPGSVGGLSPSQASSAASSASSSPGSGISEALRAGAGSGTGYNKEFLLYLAGFVDGDGSIYATIQPTQCAKFKHQLTLRFSVSQKTQRRWFLDKLVDEIGVGYVCDKGSVSEYMLSEIKPLHNFLTQLQPFLKLKQKQANLVLKIIEQLPSAKESPDKFLEVCTWVDQIAALNDSKTRKTTSETVRAVLDSLSEKKKSSP

SEQ ID NO: 138 - protein, 364 aa, synthetic construct
  REGION 1..364: note = Description of Artificial Sequence: Syntheticpolypeptide
MAPKKKRKVHMNTKYNKEFLLYLAGFVDGDGSIYACILPVQRCKFKHGLSLRFMVSQKTQRRWFLDKLVDEIGVGYVYDCGSVSEYRLSEIKPLHNFLTQLQPFLKLKQKQANLVLKIIEQLPSAKESPDKFLEVCTWVDQIAALNDSKTRKTTSETVRAVLDSLPGSVGGLSPSQASSAASSASSSPGSGISEALRAGAGSGTGYNKEFLLYLAGFVDGDGSIFASIVPDQRSKFKHGLALRFNVVQKTQRRWFLDKLVDEIGVGYVYDQGSVSEYRLSEIKPLHNFLTQLQPFLKLKQKQANLVLKIIEQLPSAKESPDKFLEVCTWVDQIAALNDSKTRKTTSETVRAVLDSLSEKKKSSP

SEQ ID NO: 139 - DNA, 1791 bp, synthetic construct
  misc_feature 1..1791: note = Description of Artificial Sequence: Syntheticpolynucleotide
  source 1..1791: mol_type = other DNA
cacaggtgtccactcccagttcaattacagctcttaaggctagagtacttaatacgactcactataggctagcctcgagccgccaccatggcaccgaagaagaagcgcaaggtgcatatgaatacaaaatataataaagagttcttactctacttagcagggtttgtagacggtgacggttccatctatgcctggatcagtccttcgcaaacgtgtaagttcaagcacaggctgatgctccggttcattgtctcgcagaagacacagcgccgttggttcctcgacaagctggtggacgagatcggtgtgggttacgtgcaggactgtggcagcgtctccgagtaccggctgtccgagatcaagcctttgcataattttttaacacaactacaaccttttctaaaactaaaacaaaaacaagcaaatttagttttaaaaattattgaacaacttccgtcagcaaaagaatccccggacaaattcttagaagtttgtacatgggtggatcaaattgcagctctgaatgattcgaagacgcgtaaaacaacttctgaaaccgttcgtgctgtgctagacagtttaccaggatccgtgggaggtctatcgccatctcaggcatccagcgccgcatcctcggcttcctcaagcccgggttcagggatctccgaagcactcagagctggagcaggttccggcactggatacaacaaggaattcctgctctacctggcgggcttcgtcgacggggacggctccatctatgcctgtatccttccgactcagcgtcagaagttcaagcacgggctgacgctctatttccgggtcactcagaagacacagcgccgttggttcctcgacaagctggtggacgagatcggtgtgggttacgtgctggactttggcagcgtctcctgttactctctgtcccagatcaagcctctgcacaacttcctgacccagctccagcccttcctgaagctcaagcagaagcaggccaacctcgtgctgaagatcatcgagcagctgccctccgccaaggaatccccggacaagttcctggaggtgtgcacctgggtggaccagatcgccgctctgaacgactccaagacccgcaagaccacttccgaaaccgtccgcgccgttctagacagtctctccgagaagaagaagtcgtccccctaaacagtctctccgagaagaagaagtcgtccccctagcggccgcttcgagcagacatgataagatacattgatgagtttggacaaaccacaactagaatgcagtgaaaaaaatgctttatttgtgaaatttgtgatgctattgctttatttgtaaccattataagctgcaataaacaagttaacaacaacaattgcattcattttatgtttcaggttcagggggagatgtgggaggttttttaaagcaagtaaaacctctacaaatgtggtaaaatcgataagatcttgatccgggctggcgtaatagcgaagaggcccgcaccgatcgcccttcccaacagttgcgcagcctgaatggcgaatggacgcgccctgtagcggcgcattaagcgcggcgggtgtggtggttacgcgcagcgtgaccgctacacttgccagcgccctagcgcccgctcctttcgctttcttcccttcctttctcgccacgttcgccggctttccccgtcaagctctaaatcgggggctccctttagggttccgatttagtgctttacggcacctcgaccccaaaaaacttgattagggtgatggttcacgtagtgggccatcg

SEQ ID NO: 140 - DNA, 1791 bp, synthetic construct
  misc_feature 1..1791: note = Description of Artificial Sequence: Syntheticpolynucleotide
  source 1..1791: mol_type = other DNA
cacaggtgtccactcccagttcaattacagctcttaaggctagagtacttaatacgactcactataggctagcctcgagccgccaccatggcaccgaagaagaagcgcaaggtgcatatgaatacaaaatataataaagagttcttactctacttagcagggtttgtagacggtgacggttccatctttgcctctatccggcctcggcaaacgagtaagttcaagcacgcgctggctctctttttcgtggtcgggcagaagacacagcgccgttggttcctcgacaagctggtggacgagatcggtgtgggttacgtgtatgaccgtggcagcgtctccgtgtaccagctgtcccagatcaagcctttgcataattttttaacacaactacaaccttttctaaaactaaaacaaaaacaagcaaatttagttttaaaaattattgaacaacttccgtcagcaaaagaatccccggacaaattcttagaagtttgtacatgggtggatcaaattgcagctctgaatgattcgaagacgcgtaaaacaacttctgaaaccgttcgtgctgtgctagacagtttaccaggatccgtgggaggtctatcgccatctcaggcatccagcgccgcatcctcggcttcctcaagcccgggttcagggatctccgaagcactcagagctggagcaggttccggcactggatacaacaaggaattcctgctctacctggcgggcttcgtcgacggggacggctccatcattgcctgtatccggcctcatcaagcttataagttcaagcaccagctgtgtctctctttctgtgtctatcagaagacacagcgccgttggttcctcgacaagctggtggacgagatcggtgtgggttacgtgacggacgctggcagcgtctcctcttaccggctgtccgagatcaagcctctgcacaacttcctgacccagctccagcccttcctgaagctcaagcagaagcaggccaacctcgtgctgaagatcatcgagcagctgccctccgccaaggaatccccggacaagttcctggaggtgtgcacctgggtggaccagatcgccgctctgaacgactccaagacccgcaagaccacttccgaaaccgtccgcgccgttctagacagtctctccgagaagaagaagtcgtccccctaaacagtctctccgagaagaagaagtcgtccccctagcggccgcttcgagcagacatgataagatacattgatgagtttggacaaaccacaactagaatgcagtgaaaaaaatgctttatttgtgaaatttgtgatgctattgctttatttgtaaccattataagctgcaataaacaagttaacaacaacaattgcattcattttatgtttcaggttcagggggagatgtgggaggttttttaaagcaagtaaaacctctacaaatgtggtaaaatcgataagatcttgatccgggctggcgtaatagcgaagaggcccgcaccgatcgcccttcccaacagttgcgcagcctgaatggcgaatggacgcgccctgtagcggcgcattaagcgcggcgggtgtggtggttacgcgcagcgtgaccgctacacttgccagcgccctagcgcccgctcctttcgctttcttcccttcctttctcgccacgttcgccggctttccccgtcaagctctaaatcgggggctccctttagggttccgatttagtgctttacggcacctcgaccccaaaaaacttgattagggtgatggttcacgtagtgggccatcg

SEQ ID NO: 141 - DNA, 31 bp, synthetic construct
  misc_feature 1..31: note = Description of Artificial Sequence: Syntheticprimer
  source 1..31: mol_type = other DNA
gaaagaaaatgccaatagtccaaaatagttg

SEQ ID NO: 142 - DNA, 25 bp, synthetic construct
  misc_feature 1..25: note = Description of Artificial Sequence: Syntheticprimer
  source 1..25: mol_type = other DNA
catattcaaaggacaccacaagttg

SEQ ID NO: 143 - DNA, 1791 bp, synthetic construct
  misc_feature 1..1791: note = Description of Artificial Sequence: Syntheticpolynucleotide
  source 1..1791: mol_type = other DNA
cacaggtgtccactcccagttcaattacagctcttaaggctagagtacttaatacgactcactataggctagcctcgagccgccaccatggcaccgaagaagaagcgcaaggtgcatatgaatacaaaatataataaagagttcttactctacttagcagggtttgtagacggtgacggttccatctttgcctgtatccagcctgatcaaagggcgaagttcaagcacacgctgcggctctctttcgaggtcgggcagaagacacagcgccgttggttcctcgacaagctggtggacgagatcggtgtgggttacgtgaatgactctggcagcgtctccaagtacaggctgtcccagatcaagcctttgcataattttttaacacaactacaaccttttctaaaactaaaacaaaaacaagcaaatttagttttaaaaattattgaacaacttccgtcagcaaaagaatccccggacaaattcttagaagtttgtacatgggtggatcaaattgcagctctgaatgattcgaagacgcgtaaaacaacttctgaaaccgttcgtgctgtgctagacagtttaccaggatccgtgggaggtctatcgccatctcaggcatccagcgccgcatcctcggcttcctcaagcccgggttcagggatctccgaagcactcagagctggagcaggttccggcactggatacaacaaggaattcctgctctacctggcgggcttcgtcgacggggacggctccatctatgccactatccagcctactcaatgtgcgaagttcaagcaccagctgactctccgtttctcggtctctcagaagacacagcgccgttggttcctcgacaagctggtggacgagatcggtgtgggttacgtgtgtgacaagggcagcgtctccgagtacatgctgtccgagatcaagcctctgcacaacttcctgacccagctccagcccttcctgaagctcaagcagaagcaggccaacctcgtgctgaagatcatcgagcagctgccctccgccaaggaatccccggacaagttcctggaggtgtgcacctgggtggaccagatcgccgctctgaacgactccaagacccgcaagaccacttccgaaaccgtccgcgccgttctagacagtctctccgagaagaagaagtcgtccccctaaacagtctctccgagaagaagaagtcgtccccctagcggccgcttcgagcagacatgataagatacattgatgagtttggacaaaccacaactagaatgcagtgaaaaaaatgctttatttgtgaaatttgtgatgctattgctttatttgtaaccattataagctgcaataaacaagttaacaacaacaattgcattcattttatgtttcaggttcagggggagatgtgggaggttttttaaagcaagtaaaacctctacaaatgtggtaaaatcgataagatcttgatccgggctggcgtaatagcgaagaggcccgcaccgatcgcccttcccaacagttgcgcagcctgaatggcgaatggacgcgccctgtagcggcgcattaagcgcggcgggtgtggtggttacgcgcagcgtgaccgctacacttgccagcgccctagcgcccgctcctttcgctttcttcccttcctttctcgccacgttcgccggctttccccgtcaagctctaaatcgggggctccctttagggttccgatttagtgctttacggcacctcgaccccaaaaaacttgattagggtgatggttcacgtagtgggccatcg

SEQ ID NO: 144 - DNA, 1791 bp, synthetic construct
  misc_feature 1..1791: note = Description of Artificial Sequence: Syntheticpolynucleotide
  source 1..1791: mol_type = other DNA
cacaggtgtccactcccagttcaattacagctcttaaggctagagtacttaatacgactcactataggctagcctcgagccgccaccatggcaccgaagaagaagcgcaaggtgcatatgaatacaaaatataataaagagttcttactctacttagcagggtttgtagacggtgacggttccatctatgcctgtatcttgccggtgcagcgttgtaagttcaagcacgggctgtctctccgattcatggtcagtcagaagacacagcgccgttggttcctcgacaagctggtggacgagatcggtgtgggttacgtgtatgactgtggcagcgtctccgagtacaggctgtccgagatcaagcctttgcataattttttaacacaactacaaccttttctaaaactaaaacaaaaacaagcaaatttagttttaaaaattattgaacaacttccgtcagcaaaagaatccccggacaaattcttagaagtttgtacatgggtggatcaaattgcagctctgaatgattcgaagacgcgtaaaacaacttctgaaaccgttcgtgctgtgctagacagtttaccaggatccgtgggaggtctatcgccatctcaggcatccagcgccgcatcctcggcttcctcaagcccgggttcagggatctccgaagcactcagagctggagcaggttccggcactggatacaacaaggaattcctgctctacctggcgggcttcgtcgacggggacggctccatctttgcctctatcgtgccggatcagcgtagtaagttcaagcacggtctggctctcaggttcaatgtcgttcagaagacacagcgccgttggttcctcgacaagctggtggacgagatcggtgtgggttacgtgtatgaccagggcagcgtctccgagtacaggctgtccgagatcaagcctctgcacaacttcctgacccagctccagcccttcctgaagctcaagcagaagcaggccaacctcgtgctgaagatcatcgagcagctgccctccgccaaggaatccccggacaagttcctggaggtgtgcacctgggtggaccagatcgccgctctgaacgactccaagacccgcaagaccacttccgaaaccgtccgcgccgttctagacagtctctccgagaagaagaagtcgtccccctaaacagtctctccgagaagaagaagtcgtccccctagcggccgcttcgagcagacatgataagatacattgatgagtttggacaaaccacaactagaatgcagtgaaaaaaatgctttatttgtgaaatttgtgatgctattgctttatttgtaaccattataagctgcaataaacaagttaacaacaacaattgcattcattttatgtttcaggttcagggggagatgtgggaggttttttaaagcaagtaaaacctctacaaatgtggtaaaatcgataagatcttgatccgggctggcgtaatagcgaagaggcccgcaccgatcgcccttcccaacagttgcgcagcctgaatggcgaatggacgcgccctgtagcggcgcattaagcgcggcgggtgtggtggttacgcgcagcgtgaccgctacacttgccagcgccctagcgcccgctcctttcgctttcttcccttcctttctcgccacgttcgccggctttccccgtcaagctctaaatcgggggctccctttagggttccgatttagtgctttacggcacctcgaccccaaaaaacttgattagggtgatggttcacgtagtgggccatcg

SEQ ID NO: 145 - DNA, 23 bp, synthetic construct
  misc_feature 1..23: note = Description of Artificial Sequence: Syntheticprimer
  source 1..23: mol_type = other DNA
ctaaccgagagggtgcttttttc

SEQ ID NO: 146 - DNA, 30 bp, synthetic construct
  misc_feature 1..30: note = Description of Artificial Sequence: Syntheticprimer
  source 1..30: mol_type = other DNA
gtgtttaggtcaactaatgtgtttattttg

SEQ ID NO: 147 - protein, 364 aa, synthetic construct
  REGION 1..364: note = Description of Artificial Sequence: Syntheticpolypeptide
MAPKKKRKVHMNTKYNKEFLLYLAGFVDGDGSIFACIHPSQAYKFKHRLTLHFTVTQKTQRRWFLDKLVDEIGVGYVQDVGSVSQYRLSQIKPLHNFLTQLQPFLKLKQKQANLVLKIIEQLPSAKESPDKFLEVCTWVDQIAALNDSKTRKTTSETVRAVLDSLPGSVGGLSPSQASSAASSASSSPGSGISEALRAGAGSGTGYNKEFLLYLAGFVDGDGSISATIAPAQYGKFKHYLGLRFYVSQKTQRRWFLDKLVDEIGVGYVSDQGSVSRYCLSQIKPLHNFLTQLQPFLKLKQKQANLVLKIIEQLPSAKESPDKFLEVCTWVDQIAALNDSKTRKTTSETVRAVLDSLSEKKKSSP

SEQ ID NO: 148 - protein, 364 aa, synthetic construct
  REGION 1..364: note = Description of Artificial Sequence: Syntheticpolypeptide
MAPKKKRKVHMNTKYNKEFLLYLAGFVDGDGSIYACIRPTQSVKFKHDLLLCFDVSQKTQRRWFLDKLVDEIGVGYVYDRGSVSSYRLSEIKPLHNFLTQLQPFLKLKQKQANLVLKIIEQLPSAKESPDKFLEVCTWVDQIAALNDSKTRKTTSETVRAVLDSLPGSVGGLSPSQASSAASSASSSPGSGISEALRAGAGSGTGYNKEFLLYLAGFVDGDGSIWASIEPRQQSKFKHQLRLGFSVYQKTQRRWFLDKLVDEIGVGYVRDTGSVSCYCLSQIKPLHNFLTQLQPFLKLKQKQANLVLKIIEQLPSAKESPDKFLEVCTWVDQIAALNDSKTRKTTSETVRAVLDSLSEKKKSSP

SEQ ID NO: 149 - DNA, 22 bp, synthetic construct
  misc_feature 1..22: note = Description of Artificial Sequence: Syntheticoligonucleotide
  source 1..22: mol_type = other DNA
ttctgtgatgtgaggacatata

SEQ ID NO: 150 - DNA, 22 bp, synthetic construct
  misc_feature 1..22: note = Description of Artificial Sequence: Syntheticoligonucleotide
  source 1..22: mol_type = other DNA
actaatgaaacaccactccaca

SEQ ID NO: 151 - DNA, 26 bp, synthetic construct
  misc_feature 1..26: note = Description of Artificial Sequence: Syntheticprimer
  source 1..26: mol_type = other DNA
gtcttatcagtcaagagatcatattg

SEQ ID NO: 152 - DNA, 27 bp, synthetic construct
  misc_feature 1..27: note = Description of Artificial Sequence: Syntheticprimer
  source 1..27: mol_type = other DNA
gtgtcagtaatctctatccctttcatg

SEQ ID NO: 153 - DNA, 214 bp, Mus sp.
  source 1..214: mol_type = genomic DNA
agaatttaaatattaacaaactataacactatgattaaatgcttgatattgagtagttattttaatagcctaagtctggaaattaaatactagtaagagaaacttctagaatttaaatattaacaaactataacactatgattaaatgcttgatattgagtagttattttaatagcctaagtctggaaattaaatactagtaagagaaacttct

SEQ ID NO: 154 - DNA, 80 bp, Mus sp.
  source 1..80: mol_type = genomic DNA
tttaatagcctaagtctggaaatactccacaggtgatttcagccactttatgaactgctggaagcaaaaatgagatcttt

SEQ ID NO: 155 - DNA, 181 bp, Mus sp.
  source 1..181: mol_type = genomic DNA
ttagttagaatttaaatattaacaaactataacactatgattaaatgcttgatattgagtagttattttaatagcctaagtctggaaattaaatactagtaagagaaacttctgtgatgtgaccactccacaggtgatttcagccactttatgaactgctggaagcaaaaatgagatcttt

SEQ ID NO: 156 - DNA, 691 bp, Mus sp.
  source 1..691: mol_type = genomic DNA
tataacactatgattaaatgcttgatattgagtagttattttatgtgtcataccttcttggattgtctgtataaatgaattgattttttttcaccaactccaagtatacttaacattttaacataataatttaaaatatccttattccattatgttcattttttaagttgtagatatgatttagctcacagcatacatatatacacatgtattacatatgcatatattatatatatggcagacatatgttttcactaccatatttcacttttgaattatgaatatatgtttaatttctgccatatttccttccctacattgacttctattaatttagtatttcagtagttctaacacattaataataacctagactcaatacagtaatctaacaattatatttgtgcctgtaattctaagttagttaaattcataggttgtgtttctcatagttggccatttgtgaaatataataatatccgaaaagaaagttcaaaaatgtcatgacttcatatagagttattgaaacagtgcccttactttcattctggccatgctagtgacttgatcattcttgtattttacagctaaaacactaccaaaagtgtcaaatccatgatctacatgtttgaccactccacaggtgatttcagccactttatgaactgctggaagcaaaaatgagatcttt

SEQ ID NO: 157 - DNA, 112 bp, Mus sp.
  source 1..112: mol_type = genomic DNA
ttgagtagttattttaatagcctaagtctggaaattaaatactagtaagagaaacttctgtgatgtgcacaggtgatttcagccactttatgaactgctggaagcaaaaatg

SEQ ID NO: 158 - DNA, 90 bp, Mus sp.
  source 1..90: mol_type = genomic DNA
gatattgagtagttattttaatagcctaagtctggaaattaaatactagtagatttcagccactttatgaactgctggaagcaaaaatga

SEQ ID NO: 159 - DNA, 182 bp, Mus sp.
  source 1..182: mol_type = genomic DNA
aatactagtaagagaaacttctgtgatgtgaggactccacaggtgatttcagccactttatgaactgctggaagcaaaaatgagatctttgcaacatgaagcagttgctcagttcattaaactgtgttcaatatttcagccataacatacattagagaatgatttatattgttcaaacattt

SEQ ID NO: 160 - DNA, 172 bp, Mus sp.
  source 1..172: mol_type = genomic DNA
aatactagtaagagaaacttctgtgatgtgaggacatttcagccactttatgaactgctggaagcaaaaatgagatctttgcaacatgaagcagttgctcagttcattaaactgtgttcaatatttcagccataacatacattagagaatgatttatattgttcaaacattt

SEQ ID NO: 161 - DNA, 154 bp, Mus sp.
  source 1..154: mol_type = genomic DNA
aatactagtaagagaagatttcagccactttatgaactgctggaagcaaaaatgagatctttgcaacatgaagcagttgctcagttcattaaactgtgttcaatatttcagccataacatacattagagaatgatttatattgttcaaacattt

SEQ ID NO: 162 - DNA, 81 bp, Mus sp.
  source 1..81: mol_type = genomic DNA
tttaatagcctaagtctggaaattaaatactagtaagagagtgatttcagccactttatgaactgctggaagcaaaaatga

SEQ ID NO: 163 - DNA, 235 bp, Mus sp.
  source 1..235: mol_type = genomic DNA
ttagttagaatttaaatattaacaaactataacactatgattaaatgcttgatattgagtagttattttaatagcctaagtctggaaattaaatactagttcagccactttatgaactgctggaagcaaaaatgagatctcattaaactgtgttcaatatttcagccataacatacattagagaatgatttatattgttcaaacatttggtgctctatttttgcatgacgtggga

SEQ ID NO: 164 - DNA, 334 bp, Mus sp.
  source 1..334: mol_type = genomic DNA
ttagttagaatttaaatattaacaaactataacactatgattaaatgcttgatattgagtagttattttaatagcctaagtctggaaattaaatactagtaagagaaacttctgtgatgtgaggacatataaagactaatttttttgttgattctaaaaatccacaggtgatttcagccactttatgaactgctggaagcaaaaatgagatctttgcaacatgaagcagttgctcagttcattaaactgtgttcaatatttcagccataacatacattagagaatgatttatattgttcaaacatttggtgctctatttttgcatgacgtggga

SEQ ID NO: 165 - DNA, 203 bp, Mus sp.
  source 1..203: mol_type = genomic DNA
ttagttagaatttaaatattaacaaactataacactatgattaaatgcttgatattgagtagttattttaatagcctaagtctggaaattaaatactagtaagagaaacttctgtgatgtgaggacatataaagactaattttttcactccacaggtgatttcagccactttatgaactgctggaagcaaaaatgagatcttt

SEQ ID NO: 166 - DNA, 478 bp, Mus sp.
  source 1..478: mol_type = genomic DNA
ttattttaatagcctaagtctggaaattaaatactagtaagagaaacttctgtgatgtgaggacatataaagactaatttttttgttgattctaaaaatcccatgttgtatacttattctttttaaatctgaaaatatattaatcatatattgcctaaatgtcttaataatgtttcactgtaggtaagttaaaatgtatcacatatataataaacatagttattaatgcatagatattcagtaaaattatgacttctaaatttctgtctaaatataatatgccctgtaatataatagaaattattcataagaatacatatatattgctttatcagatattctactttgtttagatctctaaattacataaacttttatttaccttcttcttgatatgaatgaaactcatcaaatatgcgtgttagtgtaaatgaacttctatttaaactccacaggtgatttcagccactttatgaac

SEQ ID NO: 167 - DNA, 703 bp, Mus sp.
  source 1..703: mol_type = genomic DNA
ttagttagaatttaaatattaacaaactataacactatgattaaatgcttgatattgagtagttattttaatagcctaagtctggaaattaaatactagtaagagaaacttctgtgatgtgaggacatataaagactaatttttttgttgattctaaaaatcccatgttgtatacttattctttttaaatctgaaaatatattaatcatatattgcctaaatgtcttaataatgtttcactgtaggtaagttaaaatgtatcacatatataataaacatagttattaatgcatagatattcagtaaaattatgacttctaaatttctgtctaaatataatatgccctgtaatataatagaaattattcataagaatacatatatattgctttatcagatattctactttgtttagatctctaaattacataaacttttatttaccttcttcttgatatgaatgaaactcatcaaatatgcgtgttagtgtaaatgaacttctatttaattttgaggctctgcaaagttctccacaggtgatttcagccactttatgaactgctggaagcaaaaatgagatctttgcaacatgaagcagttgctcagttcattaaactgtgttcaatatttcagccataacatacattagagaatgatttatattgttcaaacatttggtgctctatttttgcatgacgtggga

SEQ ID NO: 168 - DNA, 615 bp, Mus sp.
  source 1..615: mol_type = genomic DNA
aatactagtaagagaaacttctgtgatgtgaggacatataaagactaatttttttgttgattctaaaaatcccatgttgtatacttattctttttaaatctgaaaatatattaatcatatattgcctaaatgtcttaataatgtttcactgtaggtaagttaaaatgtatcacatatataataaacatagttattaatgcatagatattcagtaaaattatgacttctaaatttctgtctaaatataatatgccctgtaatataatagaaattattcataagaatacatatatattgctttatcagatattctactttgtttagatctctaaattacataaacttttatttaccttcttcttgatatgaatgaaactcatcaaatatgcgtgttagtgtaaatgaacttctatttaattttgaggctctgcaaagttctttgaaagagcaacaaaatggcttcaccactccacaggtgatttcagccactttatgaactgctggaagcaaaaatgagatctttgcaacatgaagcagttgctcagttcattaaactgtgttcaatatttcagccataacatacattagagaatgatttatattgttcaaacattt

SEQ ID NO: 169 - DNA, 776 bp, Mus sp.
  source 1..776: mol_type = genomic DNA
ttagttagaatttaaatattaacaaactataacactatgattaaatgcttgatattgagtagttattttaatagcctaagtctggaaattaaatactagtaagagaaacttctgtgatgtgaggacatataaagactaatttttttgttgattctaaaaatcccatgttgtatacttattctttttaaatctgaaaatatattaatcatatattgcctaaatgtcttaataatgtttcactgtaggtaagttaaaatgtatcacatatataataaacatagttattaatgcatagatattcagtaaaattatgacttctaaatttctgtctaaatataatatgccctgtaatataatagaaattattcataagaatacatatatattgctttatcagatattctactttgtttagatctctaaattacataaacttttatttaccttcttcttgatatgaatgaaactcatcaaatatgcgtgttagtgtaaatgaacttctatttaattttgaggctctgcaaagttctttgaaagagcaacaaaatggcttcaactatctgagtgacactgtgaaggagatggccaagaaagcaccttcagaaatatgccatttcagccactttatgaactgctggaagcaaaaatgagatctttgcaacatgaagcagttgctcagttcattaaactgtgttcaatatttcagccataacatacattagagaatgatttatattgttcaaacatttggtgctctatttttgcatgacgtggga

SEQ ID NO: 170 - DNA, 635 bp, Mus sp.
  source 1..635: mol_type = genomic DNA
gtctggaaattaaatactagtaagagaaacttctgtgatgtgaggacatataaagactaatttttttgttgattctaaaaatcccatgttgtatacttattctttttaaatctgaaaatatattaatcatatattgcctaaatgtcttaataatgtttcactgtaggtaagttaaaatgtatcacatatataataaacatagttattaatgcatagatattcagtaaaattatgacttctaaatttctgtctaaatataatatgccctgtaatataatagaaattattcataagaatacatatatattgctttatcagatattctactttgtttagatctctaaattacataaacttttatttaccttcttcttgatatgaatgaaactcatcaaatatgcgtgttagtgtaaatgaacttctatttaattttgaggctctgcaaagttctttgaaagagcaacaaaatggcttcaactatctgagtgacactgtgaaggagatggccaagaaagcaccttcagaaatatgccagaaatatctgtcagaatttgaagagattgaggggcactggaagaaactttcctcccagttggtggaaaacaccactccacaggtgatttcagccactttat

SEQ ID NO: 171 - DNA, 714 bp, Mus sp.
  source 1..714: mol_type = genomic DNA
tggaaattaaatactagtaagagaaacttctgtgatgtgaggacatataaagactaatttttttgttgattctaaaaatcccatgttgtatacttattctttttaaatctgaaaatatattaatcatatattgcctaaatgtcttaataatgtttcactgtaggtaagttaaaatgtatcacatatataataaacatagttattaatgcatagatattcagtaaaattatgacttctaaatttctgtctaaatataatatgccctgtaatataatagaaattattcataagaatacatatatattgctttatcagatattctactttgtttagatctctaaattacataaacttttatttaccttcttcttgatatgaatgaaactcatcaaatatgcgtgttagtgtaaatgaacttctatttaattttgaggctctgcaaagttctttgaaagagcaacaaaatggcttcaactatctgagtgacactgtgaaggagatggccaagaaagcaccttcagaaatatgccagaaatatctgtcagaatttgaagagattgaggggcactggaagaaactttcctcccagttggtggaaagctgccaaaagctagaagaacatatgaataaacttcgaaaatttcaggtaagccgaggtttggcctttaaactatatttttccactccacaggtgatttcagccactttatgaac

SEQ ID NO: 172 - DNA, 1322 bp, Mus sp.
  source 1..1322: mol_type = genomic DNA
cctaagtctggaaattaaatactagtaagagaaacttctgtgatgtgaggacatataaagactaatttttttgttgattctaaaaatcccatgttgtatacttattctttttaaatctgaaaatatattaatcatatattgcctaaatgtcttaataatgtttcactgtaggtaagttaaaatgtatcacatatataataaacatagttattaatgcatagatattcagtaaaattatgacttctaaatttctgtctaaatataatatgccctgtaatataatagaaattattcataagaatacatatatattgctttatcagatattctactttgtttagatctctaaattacataaacttttatttaccttcttcttgatatgaatgaaactcatcaaatatgcgtgttagtgtaaatgaacttctatttaattttgaggctctgcaaagttctttgaaagagcaacaaaatggcttcaactatctgagtgacactgtgaaggagatggccaagaaagcaccttcagaaatatgccagaaatatctgtcagaatttgaagagattgaggggcactggaagaaactttcctcccagttggtggaaagctgccaaaagctagaagaacatatgaataaacttcgaaaatttcaggtaagccgaggtttggcctttaaactatattttttcacatagcaattaattggaaaatgtgatgggaaacagatattttacccagagtccttcaaagatattgatgatatcaaaagccaaatctatttcaaaggattgcaacttgcctatttttcctatgaaaacagtaatgtgtcataccttcttggattgtctgtataaatgaattgattttttttcaccaactccaagtatacttaacattttaacataataatttaaaatatccttattccattatgttcattttttaagttgtagatatgatttagctcacagcatacatatatacacatgtattacatatgcatatattatatatatggcagacatatgttttcactaccatatttcacttttgaattatgaatatatgtttaatttctgccatatttccttccctacattgacttctattaatttagtatttcagtagttctaacacattaataataacctagactcaatacagtaatctaacaattatatttgtgcctgtaattctaagttagttaaattcataggttgtgtttctcatagttggccatttgtgaaatataataatatccgaaaagaaagttcaaaaatgtcatgacttcatatagacaggtgatttcagccactttatg

SEQ ID NO: 173 - DNA, 6948 bp, synthetic construct
  misc_feature 1..6948: note = Description of Artificial Sequence: Syntheticpolynucleotide
  source 1..6948: mol_type = other DNA
gggggggggggggggggttggccactccctctctgcgcgctcgctcgctcactgaggccgggcgaccaaaggtcgcccgacgcccgggctttgcccgggcggcctcagtgagcgagcgagcgcgcagagagggagtggccaactccatcactaggggttcctagatcttcaatattgggtattagtcatcgctattaccatgatgatgcggttttggcagtacaccaatgggcgtggatagcggtttgactcacggggatttccaagtctccaccccattgacgtcaatgggagtttgttttggcaccaaaatcaacgggactttccaaaatgtcgtaataaccccgccccgttgacgcaaatgggcggtaggcgtgtacggtgggaggtctatataagcagagctcgtttagtgaaccgtcagatcactagaagctttattgcggtagtttatcacagttaaattgctagcgcagtcagtgcttctgacacaacagtctcgaacttaagctgcagaagttggtcgtgaggcactgggcaggtaagtatcaaggttacaagacaggtttaaggacaccaatagaaactgggcttgtcgagacagagaagactcttgcgtttctgataggcacctattggtcttactgacatccactttgcctttctctccacaggtaattgtgagcggataacaattgatgtcgcacaggccacggattaggcaccccaggcttgacactttatgcttccggctcgtatattgtgtggaattgtgagcggataacaatttcacacaggagatatatatatgggctaggccaccatggcaccgaagaagaagcgcaaggtgcatatgaatacaaaatataataaagagttcttactctacttagcagggtttgtagacggtgacggttccatctttgcctgtatccatcctagtcaagcgtataagttcaagcaccggctgactctccatttcacggtcactcagaagacacagcgccgttggttcctcgacaagctggtggacgagatcggtgtgggttacgtgcaggacgtgggcagcgtctcccagtaccggctgtcccagatcaagcctttgcataattttttaacacaactacaaccttttctaaaactaaaacaaaaacaagcaaatttagttttaaaaattattgaacaacttccgtcagcaaaagaatccccggacaaattcttagaagtttgtacatgggtggatcaaattgcagctctgaatgattcgaagacgcgtaaaacaacttctgaaaccgttcgtgctgtgctagacagtttaccaggatccgtgggaggtctatcgccatctcaggcatccagcgccgcatcctcggcttcctcaagcccgggttcagggatctccgaagcactcagagctggagcaggttccggcactggatacaacaaggaattcctgctctacctggcgggcttcgtcgacggggacggctccatctctgccactatcgctccggctcagtatggtaagttcaagcactatctggggctccggttctatgtcagtcagaagacacagcgccgttggttcctcgacaagctggtggacgagatcggtgtgggttacgtgagtgaccagggcagcgtctccaggtactgtctgtcccagatcaagcctctgcacaacttcctgacccagctccagcccttcctgaagctcaagcagaagcaggccaacctcgtgctgaagatcatcgagcagctgccctccgccaaggaatccccggacaagttcctggaggtgtgcacctgggtggaccagatcgccgctctgaacgactccaagacccgcaagaccacttccgaaaccgtccgcgccgttctagacagtctctccgagaagaagaagtcgtccccctaaggtaccagcggccgcttcgagcagacatgataagatacattgatgagtttggacaaaccacaactagaatgcagtgaaaaaaatgctttatttgtgaaatttgtgatgctattgctttatttgtaaccattataagctgcaataaacaagttgtattagtcatcgctattaccatgatgatgcggttttggcagtacaccaatgggcgtggatagcggtttgactcacggggatttccaagtctccaccccattgacgtcaatgggagtttgttttggcaccaaaatcaacgggactttccaaaatgtcgtaataaccccgccccgttgacgcaaatgggcggtaggcgtgtacggtgggaggtctatataagcagagctcgtttagtgaaccgtcagatcactagaagctttattgcggtagtttatcacagttaaattgctagcgcagtcagtgcttctgacacaacagtctcgaacttaagctgcagaagttggtcgtgaggcactgggcaggtaagtatcaaggttacaagacaggtttaaggacaccaatagaaactgggcttgtcgagacagagaagactcttgcgtttctgataggcacctattggtcttactgacatccactttgcctttctctccacaggtaattgtgagcggataacaattgatgtcgcacaggccacggattaggcaccccaggcttgacactttatgcttccggctcgtatattgtgtggaattgtgagcggataacaatttcacacaggagatatatatatgggctaggccaccatggcaccgaagaagaagcgcaaggtgcatatgaatacaaaatataataaagagttcttactctacttagcagggtttgtagacggtgacggttccatctatgcctgtatcaggccgacgcagagtgtgaagttcaagcacgatctgctgctctgtttcgatgtctctcagaagacacagcgccgttggttcctcgacaagctggtggacgagatcggtgtgggttacgtgtatgaccgtggcagcgtctcctcgtacaggctgtccgagatcaagcctttgcataattttttaacacaactacaaccttttctaaaactaaaacaaaaacaagcaaatttagttttaaaaattattgaacaacttccgtcagcaaaagaatccccggacaaattcttagaagtttgtacatgggtggatcaaattgcagctctgaatgattcgaagacgcgtaaaacaacttctgaaaccgttcgtgctgtgctagacagtttaccaggatccgtgggaggtctatcgccatctcaggcatccagcgccgcatcctcggcttcctcaagcccgggttcagggatctccgaagcactcagagctggagcaggttccggcactggatacaacaaggaattcctgctctacctggcgggcttcgtcgacggggacggctccatctgggcctcgatcgagcctaggcaacagtctaagttcaagcaccagctgcggctcgggttctcggtctatcagaagacacagcgccgttggttcctcgacaagctggtggacgagatcggtgtgggttacgtgcgtgacactggcagcgtctcctgttactgtctgtcccagatcaagcctctgcacaacttcctgacccagctccagcccttcctgaagctcaagcagaagcaggccaacctcgtgctgaagatcatcgagcagctgccctccgccaaggaatccccggacaagttcctggaggtgtgcacctgggtggaccagatcgccgctctgaacgactccaagacccgcaagaccacttccgaaaccgtccgcgccgttctagacagtctctccgagaagaagaagtcgtccccctaaggtaccagcggccgcttcgagcagacatgataagatacattgatgagtttggacaaaccacaactagaatgcagtgaaaaaaatgctttatttgtgaaatttgtgatgctattgctttatttgtaaccattataagctgcaataaacaagttaacaacaacaattgcattcattttatgtttcaggttcagggggagatgtgggaggttttttaaagcaagtaaaacctctacaaatgtggtaaaatcgataaggatctaggaacccctagtgatggagttggccactccctctctgcgcgctcgctcgctcactgaggccgcccgggcaaagcccgggcgtcgggcgacctttggtcgcccggcctcagtgagcgagcgagcgcgcagagagggagtggccaacccccccccccccccccctgcagcctggcgtaatagcgaagaggcccgcaccgatcgcccttcccaacagttgcgtagcctgaatggcgaatggcgcgacgcgccctgtagcggcgcattaagcgcggcgggtgtggtggttacgcgcagcgtgaccgctacacttgccagcgccctagcgcccgctcctttcgctttcttcccttcctttctcgccacgttcgccggctttccccgtcaagctctaaatcgggggctccctttagggttccgatttagtgctttacggcacctcgaccccaaaaaacttgattagggtgatggttcacgtagtgggccatcgccctgatagacggtttttcgccctttgacgttggagtccacgttctttaatagtggactcttgttccaaactggaacaacactcaaccctatctcggtctattcttttgatttataagggattttgccgatttcggcctattggttaaaaaatgagctgatttaacaaaaatttaacgcgaattttaacaaaatattaacgtttacaatttcctgatgcgctattttctccttacgcatctgtgcggtatttcacaccgcatatggtgcactctcagtacaatctgctctgatgccgcatagttaagccagccccgacacccgccaacacccgctgacgcgccctgacgggcttgtctgctcccggcatccgcttacagacaagctgtgaccgtctccgggagctgcatgtgtcagaggttttcaccgtcatcaccgaaacgcgcgagacgaaagggcctcgtgatacgcctatttttataggttaatgtcatgataataatggtttcttagacgtcaggtggcacttttcggggaaatgtgcgcggaacccctatttgtttatttttctaaatactttcaaatatgtatccgctcatgagacaataaccctgataaatgcttcaataatattgaaaaaggaagagtatgagtattcaacatttccgtgtcgcccttattcccttttttgcggcattttgccttcctgtttttgctcacccagaaacgctggtgaaagtaaaagatgctgaagatcagttgggtgcacgagtgggttacatcgaactggatctcaacagcggtaagatccttgagagttttcgccccgaagaacgttttccaatgatgagcacttttaaagttctgctatgtggcgcggtattatcccgtattgacgccgggcaagagcaactcggtcgccgcatacactattctcagaatgacttggttgagtactcaccagtcacagaaaagcatcttacggatggcatgacagtaagagaattatgcagtgctgccataaccatgagtgataacactgcggccaacttacttctgacaacgatcggaggaccgaaggagctaaccgcttttttgcacaacatgggggatcatgtaactcgccttgatcgttgggaaccggagctgaatgaagccataccaaacgacgagcgtgacaccacgatgcctgtagcaatggcaacaacgttgcgcaaactattaactggcgaactacttactctagcttcccggcaacaattaatagactggatggaggcggataaagttgcaggaccacttctgcgctcggcccttccggctggctggtttattgcggataaatctggagccggtgagcgtgggtctcgcggtatcattgcagcactggggccagatggtaagccctcccgtatcgtagttatctacacgacggggagtcaggcaactatggatgaacgaaatagacagatcgctgagataggtgcctcactgattaagcattggtaactgtcagaccaagtttactcatatatactttagattgatttaaaacttcatttttaatttaaaaggatctaggtgaagatcctttttgataatctcatgaccaaaatcccttaacgtgagttttcgttccactgagcgtcagaccccgtagaaaagatcaaaggatcttcttgagatcctttttttctgcgcgtaatctgctgcttgcaaacaaaaaaaccaccgctaccagcggtggtttgtttgccggatcaagagctaccaactctttttccgaaggtaactggcttcagcagagcgcagataccaaatactgtccttctagtgtagccgtagttaggccaccacttcaagaactctgtagcaccgcctacatacctcgctctgctaatcctgttaccagtggctgctgccagtggcgataagtcgtgtcttaccgggttggactcaagacgatagttaccggataaggcgcagcggtcgggctgaacggggggttcgtgcacacagcccagcttggagcgaacgacctacaccgaactgagatacctacagcgtgagcattgagaaagcgccacgcttcccgaagggagaaaggcggacaggtatccggtaagcggcagggtcggaacaggagagcgcacgagggagcttccagggggaaacgcctggtatctttatagtcctgtcgggtttcgccacctctgacttgagcgtcgatttttgtgatgctcgtcaggggggcggagcctatggaaaaacgccagcaacgcggcctttttacggttcctggccttttgctggccttttgctcacatgttctttcctgcgttatcccctgattctgtggataaccgtattaccgcctttgagtgagctgata

SEQ ID NO: 174 - DNA, 35 bp, Mus sp.
  source 1..35: mol_type = genomic DNA
catttcatatttagtgacataagatatgaagtatg

SEQ ID NO: 175 - DNA, 27 bp, Mus sp.
  source 1..27: mol_type = genomic DNA
gtgtcagtaatctctatccctttcatg

SEQ ID NO: 176 - DNA, 330 bp, Mus sp.
  source 1..330: mol_type = genomic DNA
catttcatatttagtgacataagatatgaagtatgattattcagccactttatgaactgctggaagcaaaaatgagatctttgcaacatgaagcagttgctcagttcattaaactgtgttcaatatttcagccataacatacattagagaatgatttatattgttcaaacatttggtgctctatttttgcatgacgtgggattaaacacagcaccaacaatcaaacaattgcaaagatgtattacaagtattttttctttttaaaacaggaaagtatacttatatttccattgtccaaaccatcatgaaagggatagagattactgacac

SEQ ID NO: 177 - DNA, 381 bp, Mus sp.
  source 1..381: mol_type = genomic DNA
catttcatatttagtgacataagatatgaagtatgattattaaaattaaatcacattattttattataattactttactccacaggtgatttcagccactttatgaactgctggaagcaaaaatgagatctttgcaacatgaagcagttgctcagttcattaaactgtgttcaatatttcagccataacatacattagagaatgatttatattgttcaaacatttggtgctctatttttgcatgacgtgggattaaacacagcaccaacaatcaaacaattgcaaagatgtattacaagtattttttctttttaaaacaggaaagtatacttatatttccattgtccaaaccatcatgaaagggatagagattactgacac

SEQ ID NO: 178 - DNA, 378 bp, Mus sp.
  source 1..378: mol_type = genomic DNA
catttcatatttagtgacataagatatgaagtatgattattaaaattaaatcacattattttattataattactttacacaggtgatttcagccactttatgaactgctggaagcaaaaatgagatctttgcaacatgaagcagttgctcagttcattaaactgtgttcaatatttcagccataacatacattagagaatgatttatattgttcaaacatttggtgctctatttttgcatgacgtgggattaaacacagcaccaacaatcaaacaattgcaaagatgtattacaagtattttttctttttaaaacaggaaagtatacttatatttccattgtccaaaccatcatgaaagggatagagattactgacac

SEQ ID NO: 179 - DNA, 1083 bp, synthetic construct
  misc_feature 1..1083: note = Description of Artificial Sequence: Syntheticpolynucleotide
  source 1..1083: mol_type = other DNA
gaaagaaaatgccaatagtccaaaatagttgctttatctttcttttaatcaataaatatattcattttaaagggaaaaattgcaaccttccatttaaaatcagcttttatattgagtatttttttaaaatgttgtgtgtacatgctaggtgtgtatattaatttttatttgttacttgaaactaaactctgcaaatgcaggaaactatcagagtgatatctttgtcagtataaccaaaaaatatacgctatatctctataatctgttttacataatccatctatttttcttgatccatatgcttttacctgcaggcgatttgacagatctgttgagaaatggcggcgttttcattatgatataaagatatttaatcagtggctaacagaagctgaacagtttctcagaaagacacaaattcctgagaattgggaacatgctaaatacaaatggtatcttaaggtaagtctttgatttgttttttcgaaattgtatttatcttcagcacatctggactctttaacttcttaaagatcaggttctgaagggtgatggaaattacttttgactgttgttgtcatcattatattactagaaagaaaattatcataatgataatattagagcacggtgctatggactttttgtgtcaggatgagagagtttgcctggacggagctggtttatctgataaactgcaaaatataattgaatctgtgacagagggaagcatcgtaacagcaaggtgttttgtggctttggggcagtgtgtatttcggctttatgttggaacctttccagaaggagaacttgtggcatacttagctaaaatgaagttgctagaaatatccatcatgataaaattacagttctgttttcctaaagacaattttgtagtgctgtagcaatatttctatatattctattgacaaaatgccttctgaaatagtccagaggccaaaacaatgcagagttaattgttggtacttattgacattttatggtttatgttaatagggaaacagcatatggatgataaccagtgtgtagtttaatttcaacttgtggtgtcctttgaatatg

SEQ ID NO: 180 - DNA, 875 bp, Homo sapiens
  variation 29..846: note = a, c, t, g, unknown or other
  source 1..875: mol_type = genomic DNA
aaaatgttgtgtgtacatgctaggtgtgnnnnnnnnnnnnnnnnnnnnnnnnnnnnnnnnnnnnnnnnnnnnnnnnnnnnnnnnnnnnnnnnnnnnnnnnnnnnnnnnnnnnnnnnnnnnnnnnnnnnnnnnnnnnnnnnnnnnnnnnnnnnnnnnnnnnnnnnnnnnnnnnnnnnnnnnnnnnnnnnnnnnnnnnnnnnnnnnnnnnnnnnnnnnnnnnnnnnnnnnnnnnnnnnnnnnnnnnnnnnnnnnnnnnnnnnnnnnnnnnnnnnnnnnnnnnnnnnnnnnnnnnnnnnnnnnnnnnnnnnnnnnnnnnnnnnnnnnnnnnnnnnnnnnnnnnnnnnnnnnnnnnnnnnnnnnnnnnnnnnnnnnnnnnnnnnnnnnnnnnnnnnnnnnnnnnnnnnnnnnnnnnnnnnnnnnnnnnnnnnnnnnnnnnnnnnnnnnnnnnnnnnnnnnnnnnnnnnnnnnnnnnnnnnnnnnnnnnnnnnnnnnnnnnnnnnnnnnnnnnnnnnnnnnnnnnnnnnnnnnnnnnnnnnnnnnnnnnnnnnnnnnnnnnnnnnnnnnnnnnnnnnnnnnnnnnnnnnnnnnnnnnnnnnnnnnnnnnnnnnnnnnnnnnnnnnnnnnnnnnnnnnnnnnnnnnnnnnnnnnnnnnnnnnnnnnnnnnnnnnnnnnnnnnnnnnnnnnnnnnnnnnnnnnnnnnnnnnnnnnnnnnnnnnnnnnnnnnnnnnnnnnnnnnnnnnnnnnnnnnnnnnnnnnnnnnnnnnnnnnnnnnnnnnnnnnnnnnnnnnnnnnnnnnnnnnnnnnnnnnnnnnnnnnnnnnnnnnnnnnnnnnnnnnnnnnnnnnnnagttaattgttggtacttattgacatttt

SEQ ID NO: 181 - DNA, 29 bp, synthetic construct
  misc_feature 1..29: note = Description of Artificial Sequence: Syntheticoligonucleotide
  source 1..29: mol_type = other DNA
aaaatgttgtgtgtacttattgacatttt

SEQ ID NO: 182 - DNA, 29 bp, synthetic construct
  misc_feature 1..29: note = Description of Artificial Sequence: Syntheticoligonucleotide
  source 1..29: mol_type = other DNA
aaaatgttgtgtgtacttattgacatttt

SEQ ID NO: 183 - DNA, 19 bp, synthetic construct
  misc_feature 1..19: note = Description of Artificial Sequence: Syntheticoligonucleotide
  source 1..19: mol_type = other DNA
aaaatgttattgacatttt

SEQ ID NO: 184 - DNA, 1384 bp, synthetic construct
  misc_feature 1..1384: note = Description of Artificial Sequence: Syntheticpolynucleotide
  source 1..1384: mol_type = other DNA
ctaaccgagagggtgcttttttccctgacacataaaaggtgtctttctgtcttgtatcctttggatatgggcatgtcagtttcatagggaaattttcacatggagcttttgtatttctttctttgccagtacaactgcatgtggtagcacactgtttaatcttttctcaaataaaaagacatggggcttcatttttgttttgcctttttggtatcttacaggaactccaggatggcattgggcagcggcaaactgttgtcagaacattgaatgcaactggggaagaaataattcagcaatcctcaaaaacagatgccagtattctacaggaaaaattgggaagcctgaatctgcggtggcaggaggtctgcaaacagctgtcagacagaaaaaagaggtagggcgacagatctaataggaatgaaaacattttagcagactttttaagctttctttagaagaatatttcatgagagattataagcagggtgaaaggcactaacattaaagaacctatcaaccattaatcaacagcagtaaagaaattttttatttctttttttcatatactaaaatatatacttgtggctagttagtggttttctgctattttaaacttgaagtttgctttaaaaatcacccatgattgcttaaaggtgaatatcttcaatatattttaacttcaacaagctgaatctcagttgtttttcaagaagattttagaaagcaattataaatgattgttttgtaggaaagacagatctttgcttagttttaaaaatagctatgaatatgactatgaagctaaaaaaagtgatagtgtcacttacctctagtttcaccacatttgtgaatacattcttgaaggggaacttgagccaaagaggtacaagtttaatggggaaaacaaaacctcaaaaaggttactgtcaaattcaatcatcatttaaatttcccttggaatgtattgaaggcacagaaagccaaatgcgtgctgctgcagttggaaagcctagagagtttataaatgggattttgtattatgcttccagttgttgatgttaatgtgtcttgtttcgtaaaggaagacttggcctttatttaccaaatgagactattgttatgaacaatgaaaacttcgttcttttgccaagctcttgcatcccacccatcatccacataataggtggattttaatattcaggaagctagaacaactcattgatgaatatctttcgttaagatgtattaaaaagaagattttggaattatgtcagttgtctttgcccacctcctctttccctctttattcatgttacattattcagaaagtagatacaattcatattttgtacaaaataaacacattagttgacctaaacac

SEQ ID NO: 185 - DNA, 1253 bp, Homo sapiens
  variation 29..1223: note = a, c, t, g, unknown or other
  source 1..1253: mol_type = genomic DNA
ctttctttgccagtacaactgcatgtggnnnnnnnnnnnnnnnnnnnnnnnnnnnnnnnnnnnnnnnnnnnnnnnnnnnnnnnnnnnnnnnnnnnnnnnnnnnnnnnnnnnnnnnnnnnnnnnnnnnnnnnnnnnnnnnnnnnnnnnnnnnnnnnnnnnnnnnnnnnnnnnnnnnnnnnnnnnnnnnnnnnnnnnnnnnnnnnnnnnnnnnnnnnnnnnnnnnnnnnnnnnnnnnnnnnnnnnnnnnnnnnnnnnnnnnnnnnnnnnnnnnnnnnnnnnnnnnnnnnnnnnnnnnnnnnnnnnnnnnnnnnnnnnnnnnnnnnnnnnnnnnnnnnnnnnnnnnnnnnnnnnnnnnnnnnnnnnnnnnnnnnnnnnnnnnnnnnnnnnnnnnnnnnnnnnnnnnnnnnnnnnnnnnnnnnnnnnnnnnnnnnnnnnnnnnnnnnnnnnnnnnnnnnnnnnnnnnnnnnnnnnnnnnnnnnnnnnnnnnnnnnnnnnnnnnnnnnnnnnnnnnnnnnnnnnnnnnnnnnnnnnnnnnnnnnnnnnnnnnnnnnnnnnnnnnnnnnnnnnnnnnnnnnnnnnnnnnnnnnnnnnnnnnnnnnnnnnnnnnnnnnnnnnnnnnnnnnnnnnnnnnnnnnnnnnnnnnnnnnnnnnnnnnnnnnnnnnnnnnnnnnnnnnnnnnnnnnnnnnnnnnnnnnnnnnnnnnnnnnnnnnnnnnnnnnnnnnnnnnnnnnnnnnnnnnnnnnnnnnnnnnnnnnnnnnnnnnnnnnnnnnnnnnnnnnnnnnnnnnnnnnnnnnnnnnnnnnnnnnnnnnnnnnnnnnnnnnnnnnnnnnnnnnnnnnnnnnnnnnnnnnnnnnnnnnnnnnnnnnnnnnnnnnnnnnnnnnnnnnnnnnnnnnnnnnnnnnnnnnnnnnnnnnnnnnnnnnnnnnnnnnnnnnnnnnnnnnnnnnnnnnnnnnnnnnnnnnnnnnnnnnnnnnnnnnnnnnnnnnnnnnnnnnnnnnnnnnnnnnnnnnnnnnnnnnnnnnnnnnnnnnnnnnnnnnnnnnnnnnnnnnnnnnnnnnnnnnnnnnnnnnnnnnnnnnnnnnnnnnnnnnnnnnnnnnnnnnnnnnnnnnnnnnnnnnnnnnnnnnnnnnnnnnnnnnnnnnnnnnnnnnnnnnnnnnnnnnnnnnnnnnnnnnnnnnnnnnnnnnnnnnnnnnnnnnnnnnnnnnnnnnnnnnnnnnnnnnaattcatattttgtacaaaataaacacatt

SEQ ID NO: 186 - DNA, 30 bp, synthetic construct
  misc_feature 1..30: note = Description of Artificial Sequence: Syntheticoligonucleotide
  source 1..30: mol_type = other DNA
ctttctttgccagtacaaaataaacacatt

SEQ ID NO: 187 - DNA, 15 bp, synthetic construct
  misc_feature 1..15: note = Description of Artificial Sequence: Syntheticoligonucleotide
  source 1..15: mol_type = other DNA
caaaataaacacatt

SEQ ID NO: 188 - protein, 9 aa, Homo sapiens
LAGLIDADG